European Patent Application EP 4 219 462 A1, published August 2, 2023. Title: METHODS, COMPOSITIONS AND KITS FOR INCREASING GENOME EDITING EFFICIENCY. Applicant: VERTEX PHARMACEUTICALS INCORPORATED. Application WO PCT/US17/41979, filed July 13, 2017. The sequence listing filed with the application follows.

SEQUENCE LISTING (7 sequences)

SEQ ID NO: 1 - DNA, 3531 bp, synthetic construct
  misc_feature 1..3531: note = Synthetic Polynucleotide
  source 1..3531: mol_type = other DNA
tcgcgcgtttcggtgatgacggtgaaaacctctgacacatgcagctcccggagacggtcacagcttgtctgtaagcggatgccgggagcagacaagcccgtcagggcgcgtcagcgggtgttggcgggtgtcggggctggcttaactatgcggcatcagagcagattgtactgagagtgcaccatatgcggtgtgaaataccgcacagatgcgtaaggagaaaataccgcatcaggcgccattcgccattcaggctgcgcaactgttgggaagggcgatcggtgcgggcctcttcgctattacgccagctggcgaaagggggatgtgctgcaaggcgattaagttgggtaacgccagggttttcccagtcacgacgttgtaaaacgacggccagtgaaactagtgcgacgtaaacggccacaagttcagcgtgtccggcgagggcgagggcgatgccacctacggcaagctgaccctgaagttcatctgcaccaccggcaagctgcccgtgccctggcccaccctcgtgaccaccctgacctacggcgtgcagtgcttcagccgctaccccgaccacatgaagcagcacgacttcttcaagtccgccatgcccgaaggctacgtccaggagcgcaccatcttcttcaaggacgacggcaactacaagacccgcgccgaggtgaagttcgagggcgacaccctggtgaaccgcatcgagctgaagggcatcgacttcaaggaggacggcaacatcctggggcacaagctggagtacaactacaacagccacaacgtctatatcatggccgacaagcagaagaacggcatcaaggtgaacttcaagatccgccacaacatcgaggacggcagcgtgcagctcgccgaccactaccagcagaacacccccatcggcgacggccccgtgctgctgcccgacaaccactacctgagcacccagtccgccctgagcaaagaccccaacgagaagcgcgatcacatggtcctgctggagttcgtgaccgccgccgggatcactctcggcatggacgtcgacaccggtgatatcaagcttggcgtaatcatggtcatagctgtttcctgtgtgaaattgttatccgctcacaattccacacaacatacgagccggaagcataaagtgtaaagcctggggtgcctaatgagtgagctaactcacattaattgcgttgcgctcactgcccgctttccagtcgggaaacctgtcgtgccagctgcattaatgaatcggccaacgcgcggggagaggcggtttgcgtattgggcgctcttccgcttcctcgctcactgactcgctgcgctcggtcgttcggctgcggcgagcggtatcagctcactcaaaggcggtaatacggttatccacagaatcaggggataacgcaggaaagaacatgtgagcaaaaggccagcaaaaggccaggaaccgtaaaaaggccgcgttgctggcgtttttccataggctccgcccccctgacgagcatcacaaaaatcgacgctcaagtcagaggtggcgaaacccgacaggactataaagataccaggcgtttccccctggaagctccctcgtgcgctctcctgttccgaccctgccgcttaccggatacctgtccgcctttctcccttcgggaagcgtggcgctttctcatagctcacgctgtaggtatctcagttcggtgtaggtcgttcgctccaagctgggctgtgtgcacgaaccccccgttcagcccgaccgctgcgccttatccggtaactatcgtcttgagtccaacccggtaagacacgacttatcgccactggcagcagccactggtaacaggattagcagagcgaggtatgtaggcggtgctacagagttcttgaagtggtggcctaactacggctacactagaagaacagtatttggtatctgcgctctgctgaagccagttaccttcggaaaaagagttggtagctcttgatccggcaaacaaaccaccgctggtagcggtggtttttttgtttgcaagcagcagattacgcgcagaaaaaaaggatctcaagaagatcctttgatcttttctacggggtctgacgctcagtggaacgaaaactcacgttaagggattttggtcatgagattatcaaaaaggatcttcacctagatccttttgatccccgccacggttgatgagagctttgttgtaggtggaccagttggtgattttgaacttttgctttgccacggaacggtctgcgttgtcgggaagatgcgtgatctgatccttcaactcagcaaaagttcgatttattcaacaaagccgccgtcccgtcaagtcagcgtaatgctctgccagtgttacaaccaattaaccaattctgattagaaaaactcatcgagcatcaaatgaaactgcaatttattcatatcaggattatcaataccatatttttgaaaaagccgtttctgtaatgaaggagaaaactcaccgaggcagttccataggatggcaagatcctggtatcggtctgcgattccgactcgtccaacatcaatacaacctattaatttcccctcgtcaaaaataaggttatcaagtgagaaatcaccatgagtgacgactgaatccggtgagaatggcaaaagtttatgcatttctttccagacttgttcaacaggccagccattacgctcgtcatcaaaatcactcgcatcaaccaaaccgttattcattcgtgattgcgcctgagcgagacgaaatacgcgatcgctgttaaaaggacaattacaaacaggaatcgaatgcaaccggcgcaggaacactgccagcgcatcaacaatattttcacctgaatcaggatattcttctaatacctggaatgctgtttttccggggatcgcagtggtgagtaaccatgcatcatcaggagtacggataaaatgcttgatggtcggaagaggcataaattccgtcagccagtttagtctgaccatctcatctgtaacatcattggcaacgctacctttgccatgtttcagaaacaactctggcgcatcgggcttcccatacaatcgatagattgtcgcacctgattgcccgacattatcgcgagcccatttatacccatataaatcagcatccatgttggaatttaatcgcggcctcgagcaagacgtttcccgttgaatatggctcataacaccccttgtattactgtttatgtaagcagacagttttattgttcatgatgatatatttttatcttgtgcaatgtaacatcagagattttgagacacaattcatcgatgatggttgagatgtgtataagagacagattattgaagcatttatcagggttattgtctcatgagcggatacatatttgaatgtatttagaaaaataaacaaataggggttccgcgcacatttccccgaaaagtgccacctgacgtctaagaaaccattattatcatgacattaacctataaaaataggcgtatcacgaggccctttcgtc

SEQ ID NO: 2 - DNA, 20 bp, synthetic construct
  misc_feature 1..20: note = Synthetic Oligonucleotide
  source 1..20: mol_type = other DNA
gtcccctccaccccacagtg

SEQ ID NO: 3 - DNA, 20 bp, synthetic construct
  misc_feature 1..20: note = Synthetic Oligonucleotide
  source 1..20: mol_type = other DNA
ggggccactagggacaggat

SEQ ID NO: 4 - DNA, 20 bp, synthetic construct
  misc_feature 1..20: note = Synthetic Oligonucleotide
  source 1..20: mol_type = other DNA
gcgacgtaaacggccacaag

SEQ ID NO: 5 - DNA, 20 bp, synthetic construct
  misc_feature 1..20: note = Synthetic Oligonucleotide
  source 1..20: mol_type = other DNA
gtccatgccgagagtgatcc

SEQ ID NO: 6 - DNA, 23 bp, synthetic construct
  misc_feature 1..23: note = Synthetic Oligonucleotide
  source 1..23: mol_type = other DNA
acttcttcaagtccgccatgccc

SEQ ID NO: 7 - DNA, 24 bp, synthetic construct
  misc_feature 1..24: note = Synthetic Oligonucleotide
  source 1..24: mol_type = other DNA
atgttgccgtcctccttgaagtcg